European Patent Application EP 4 186 923 A1, published May 31, 2023. Title: Anti-Henipavirus Monoclonal Antibody Having Broad Spectrum Neutralization Activity and Use Thereof. Applicant: ACADEMY OF MILITARY MEDICAL SCIENCE, PLA. Application CNPCT/2021/102588. The sequence listing filed with the application follows.

SEQUENCE LISTING (22 sequences)

SEQ ID NO: 1 - protein, 127 aa, Macaca mulatta
VQLQESGPGPVKPSETLSLTCTVSGGSMSRGYDWNWIRQPPGKGLEWIGYIGDDGGRSNYNPSLKSRVTISKDSSKNQFSLKLGSVSAADTAVYYCARALRAIWYNSGWFYNSLDVWGRGVLVTVSS

SEQ ID NO: 2 - DNA, 382 bp, Macaca mulatta
gtgcagctgcaggagtcgggcccagggccggtgaagccttcggagaccctgtccctcacctgcactgtctctggtggctccatgagcagaggttatgactggaactggatccgccagcccccagggaaagggctggagtggattggttatatcggtgatgatggtggcagatccaactacaacccctccctcaagagtcgagtcaccatttcaaaagactcgtccaagaaccagttctccctgaagctgggctctgtgagcgccgcggacaccgccgtgtattactgtgcgagagcgctgagggccatctggtataacagcggctggttctacaattcattggatgtctggggccggggagttctggtcaccgtctcctcag

SEQ ID NO: 3 - protein, 110 aa, Macaca mulatta
DIVLTQSPASLAVSPGQRATITCRASEGVSVFGRDLIHWYQQKPGQPPKLLIYQTSNRDTGVPARFSGSGSGTDFTLTINPVEADDAADYYCLQSKNSYSFGQGTKVEIK

SEQ ID NO: 4 - DNA, 331 bp, Macaca mulatta
gacattgtgctgacccagtctccagcctctttggccgtgtctccagggcagagggccaccatcacctgcagagccagtgagggtgtcagtgtctttggaagagacctcattcactggtatcaacagaaaccaggacaacctcctaaactcctgatttatcaaacatccaatagagacactggggtcccagccaggttcagcggcagtgggtctgggaccgatttcaccctcacaattaatcctgtggaagctgacgatgctgcagattattactgtctgcagagtaagaattcgtacagttttggccaggggaccaaagtggagatcaaac

SEQ ID NO: 5 - protein, 128 aa, Macaca mulatta
VQLQESGPGVVKPSETLSLTCAVSGGSISDTYRWSWIRQPPGKGLEWIGYIYGSATSTYYNPSLSSRVTISKDMSKNQFSLNLNSVTAADTAVYYCARDYQYYYSGSYPTPHNWFDVWGPGVLVTVSS

SEQ ID NO: 6 - DNA, 384 bp, Macaca mulatta
gtgcagctgcaggagtcgggcccaggagtagtgaagccttcggagaccctgtccctcacctgcgctgtctctggtggctccatcagcgatacttatcggtggagctggatccgccagcccccagggaagggactggagtggattgggtacatctatggtagtgctacgagcacctactacaacccctccctcagcagtcgagtcaccatttcaaaagacatgtccaagaaccagttctccttgaacctgaactctgtgaccgccgcggacacggccgtgtattactgtgcgagagattaccaatattactatagtggttcttatccaaccccccacaactggttcgatgtctggggcccgggagtcctggtcaccgtctcctca

SEQ ID NO: 7 - protein, 107 aa, Macaca mulatta
DIQMTQSPSSLSASVGDRVTITCRASQGIIDYLSWYQQKPGKAPKLLISTASNLESGVPSRFSGSGSGTEFTLTISSLQPEDFATYSCLQGYTTPYTFGQGTKVEIK

SEQ ID NO: 8 - DNA, 321 bp, Macaca mulatta
gacatccagatgacccagtctccatcttccctgtctgcatcggtaggagacagagtcaccatcacttgcagggcaagtcagggcattatcgattatttaagttggtatcagcagaaaccaggaaaagcccctaagctcctgatctctactgcatccaatttggaaagcggggtcccatcaaggttcagcggcagtggatctgggacagaattcactctcaccatcagcagcctgcagcctgaagattttgcaacttattcctgtctacagggttatactaccccgtacacttttggccaggggaccaaagtggagatcaaa

SEQ ID NO: 9 - protein, 126 aa, Macaca mulatta
QVQLQESGPGLVKPSETLSLTCPVSGASISSHWWTWIRQPPGKGLEWIGEIHGNSGSTNYNPSLKSRVTISKDASKNHFSLKLSSVTAADTAVYYCARDGHLGILVVFATSRFDVWGPGVLVTVSS

SEQ ID NO: 10 - DNA, 379 bp, Macaca mulatta
caggtgcagctgcaggagtcgggcccaggactggtgaagccttcggagaccctgtccctcacctgccctgtctctggtgcctccatcagtagtcactggtggacctggatccgccagcccccagggaagggactggagtggattggggagatccatggtaatagtgggagcaccaactacaacccctccctcaagagtcgagtcaccatttcaaaagacgcgtccaagaaccacttctccctgaagctgagctctgtgaccgccgcggacacggccgtgtattattgtgcgagagatgggcaccttggtattctggtggtatttgcgactagccggttcgatgtctggggcccgggagtcctggtcaccgtctcctcag

SEQ ID NO: 11 - protein, 107 aa, Macaca mulatta
DIQMTQSPSSLSASVGDTVTITCQASQGIANNLNWYQQKPGKAPKLLIYRASSLQSGIPSRFSGSGSGTDYTLTISSLQPEDFATYYCQQGYTYPRTFGQGTKVEIK

SEQ ID NO: 12 - DNA, 322 bp, Macaca mulatta
gacatccagatgacgcagtctccatcctccctgtccgcatctgtaggagacacggtcaccatcacttgccaggcgagtcaaggcattgccaataatttaaattggtatcagcagaaaccagggaaagcccctaaactcctgatctatagggcatccagtttgcaaagtgggattccctctcggttcagtggcagtggatctgggacggattacactctcaccatcagcagcctgcagcctgaagattttgccacttattactgtcaacagggttatacttaccctcggacgttcggccaagggaccaaggtggaaatcaaac

SEQ ID NO: 13 - protein, 120 aa, Macaca mulatta
VQLQESGPGLVKPSETLSLTCSVSGGSISISNWWSWIRQSPGKGLEWIGYIYGSSGSTLYNPSLKSRVSISTDTSKNQFSLKLRSVTAADTAVYYCASPSIAATGDFDYWGQGVLVTVSS

SEQ ID NO: 14 - DNA, 361 bp, Macaca mulatta
gtgcagctgcaggagtcgggcccaggactggtgaagccttcggagaccctgtccctcacctgctctgtctctggtggctccatcagcattagtaactggtggagctggatccgccagtccccagggaaggggctggagtggattggatatatctatggtagtagtgggagcaccctctacaacccctccctcaagagtcgagtctccatttcaacagacacgtccaagaaccagttttccctgaagctgaggtctgtgaccgccgcggacaccgccgtgtattactgtgcgagtccaagtatagcagcgactggggactttgactactggggccagggagtcctggtcaccgtctcctcag

SEQ ID NO: 15 - protein, 110 aa, Macaca mulatta
QSVLTQPPSASGAPGQSVTISCSGSSSNIGGNNVYWYQQLPGTAPKLLIYSSNQRPSGVPDRFSGSKSGTSASLAITGLRSEDEADYFCAVWDDSLGSPFFGGGTRLTVL

SEQ ID NO: 16 - DNA, 331 bp, Macaca mulatta
cagtctgtactgactcagccaccctcagcgtctggggctcccgggcagagtgtcaccatctcttgctctggaagcagctccaacattggaggtaataatgtatattggtaccaacagttgccaggaacggcccccaaactcctcatctattctagtaatcagcgaccctcaggagtccctgaccgattctctggctccaagtctggcacctcagcctccctggccatcactggtctccggtctgaggatgaggctgattatttctgtgcagtttgggatgacagcctgggcagtccgtttttcggaggagggacccggctgaccgtcctag

SEQ ID NO: 17 - protein, 330 aa, Homo sapiens [sequence omitted]

SEQ ID NO: 18 - DNA, 990 bp, Homo sapiens
gcctccaccaagggcccatcggtcttccccctggcaccctcctccaagagcacctctgggggcacagcagccctgggctgcctggtcaaggactacttccccgaaccggtgacggtgtcgtggaactcaggcgccctgaccagcggcgtgcacaccttcccggctgtcctacagtcctcaggactctactccctcagcagcgtggtgaccgtgccctccagcagcttgggcacccagacctacatctgcaacgtgaatcacaagcccagcaacaccaaggtggacaagaaagttgagcccaaatcttgtgacaaaactcacacatgcccaccgtgcccagcacctgaactcctggggggaccgtcagtcttcctcttccccccaaaacccaaggacaccctcatgatctcccggacccctgaggtcacatgcgtggtggtggacgtgagccacgaagaccctgaggtcaagttcaactggtacgtggacggcgtggaggtgcataatgccaagacaaagccgcgggaggagcagtacaacagcacgtaccgtgtggtcagcgtcctcaccgtcctgcaccaggactggctgaatggcaaggagtacaagtgcaaggtctccaacaaagccctcccagcccccatcgagaaaaccatctccaaagccaaagggcagccccgagaaccacaggtgtacaccctgcccccatcccgggatgagctgaccaagaaccaggtcagcctgacctgcctggtcaaaggcttctatcccagcgacatcgccgtggagtgggagagcaatgggcagccggagaacaactacaagaccacgcctcccgtgctggactccgacggctccttcttcctctacagcaagctcaccgtggacaagagcaggtggcagcaggggaacgtcttctcatgctccgtgatgcatgaggctctgcacaaccactacacacagaagagcctctccctgtctccgggtaaa

SEQ ID NO: 19 - protein, 106 aa, Homo sapiens
TVAAPSVFIFPPSDEQLKSGTASVVCLLNNFYPREAKVQWKVDNALQSGNSQESVTEQDSKDSTYSLSSTLTLSKADYEKHKVYACEVTHQGLSSPVTKSFNRGEC

SEQ ID NO: 20 - DNA, 318 bp, Homo sapiens
actgtggctgcaccatctgtcttcatcttcccgccatctgatgagcagttgaaatctggaactgcctctgttgtgtgcctgctgaataacttctatcccagagaggccaaagtacagtggaaggtggataacgccctccaatcgggtaactcccaggagagtgtcacagagcaggacagcaaggacagcacctacagcctcagcagcaccctgacgctgagcaaagcagactacgagaaacacaaagtctacgcctgcgaagtcacccatcagggcctgagttcgcccgtcacaaagagcttcaacaggggagagtgt

SEQ ID NO: 21 - protein, 106 aa, Homo sapiens [sequence omitted]

SEQ ID NO: 22 - DNA, 318 bp, Homo sapiens
cgtcagcccaaggctgccccctcggtcactctgttcccaccctcgagtgaggagcttcaagccaacaaggccacactggtgtgtctcataagtgacttctacccgggagccgtgacagtggcctggaaggcagatagcagccccgtcaaggcgggagtggagaccaccacaccctccaaacaaagcaacaacaagtacgcggccagcagctacctgagcctgacgcctgagcagtggaagtcccacaaaagctacagctgccaggtcacgcatgaagggagcaccgtggagaagacagtggcccctacagaatgttca